European Patent Specification EP 4 029 522 B1, published August 13, 2025. Title: Method for reducing immunogenicity of RNA. Applicant: BioNTech SE. The sequence listing filed with the application follows.

SEQUENCE LISTING (15 sequences)

SEQ ID NO: 1 - protein, 192 aa, Mus musculus
MGVPERPTLLLLLSLLLIPLGLPVLCAPPRLICDSRVLERYILEAKEAENVTMGCAEGPRLSENITVPDTKVNFYAWKRMEVEEQAIEVWQGLSLLSEAILQAQALLANSSQPPETLQLHIDKAISGLRSLTSLLRVLGAQKELMSPPDTTPPAPLRTLTVDTFCKLFRVYANFLRGKLKLYTGEVCRRGDR

SEQ ID NO: 2 - DNA, 579 bp, Mus musculus
atgggggtgcccgaacgtcccaccctgctgcttttactctccttgctactgattcctctgggcctcccagtcctctgtgctcccccacgcctcatctgcgacagtcgagttctggagaggtacatcttagaggccaaggaggcagaaaatgtcacgatgggttgtgcagaaggtcccagactgagtgaaaatattacagtcccagataccaaagtcaacttctatgcttggaaaagaatggaggtggaagaacaggccatagaagtttggcaaggcctgtccctgctctcagaagccatcctgcaggcccaggccctgctagccaattcctcccagccaccagagacccttcagcttcatatagacaaagccatcagtggtctacgtagcctcacttcactgcttcgggtactgggagctcagaaggaattgatgtcgcctccagataccaccccacctgctccactccgaacactcacagtggatactttctgcaagctcttccgggtctacgccaacttcctccgggggaaactgaagctgtacacgggagaggtctgcaggagaggggacaggtga

SEQ ID NO: 3 - DNA, 579 bp, Artificial Sequence
  GC-rich sequence
atgggcgtccccgaaaggcctaccctgctgctgctcctgtctctgctcctgatccccctgggactgcccgtgctgtgcgcccctcccaggctgatctgcgacagcagggtgctggaaagatacatcctggaagccaaagaggccgagaacgtcacaatgggctgcgccgagggccccagactgagcgagaacatcaccgtgcccgacaccaaggtcaacttctacgcctggaagaggatggaagtggaggaacaggccatcgaggtctggcagggactgtctctgctgtccgaggccatcctgcaggcccaggctctgctggccaattctagccagccccccgagacactgcagctgcacatcgacaaggccatcagcggcctgagaagcctgaccagcctgctgagggtgctgggagcccagaaagagctgatgagcccccctgacaccaccccccctgcccccctgaggaccctgaccgtggacaccttctgcaagctgttcagggtgtacgccaacttcctgaggggcaagctgaagctgtacaccggcgaggtctgcagacggggcgacagatga

SEQ ID NO: 4 - DNA, 579 bp, Artificial Sequence
  A-rich sequence
atgggagtgccagaaagaccaaccctgctgctgctgctcagcctgctactgatcccactgggactcccagtcctctgcgcaccaccaagactcatctgcgacagcagagtgctggaaagatacatcctagaagcaaaagaagcagaaaacgtcacgatgggatgcgcagaaggaccaagactgagcgaaaacatcacagtcccagacaccaaagtcaacttctacgcatggaaaagaatggaagtggaagaacaggcaatagaagtgtggcaaggactgagcctgctcagcgaagcaatcctgcaggcacaggcactgctagcaaacagcagccagccaccagaaaccctgcagctgcacatagacaaagcaatcagcggactaagaagcctcaccagcctgctgagagtactgggagcacagaaagaactgatgagcccaccagacaccaccccaccagcaccactcagaacactcacagtggacactttctgcaaactcttcagagtctacgcaaacttcctcagaggaaaactgaaactgtacacgggagaagtctgcagaagaggggacagatga

SEQ ID NO: 5 - DNA, 579 bp, Artificial Sequence
  Super optimized sequence
atgggagttcctgaaagaccaactctgttgctcttgctgtctttgctgctgattcctctgggtcttccggtgctttgcgcacctcccaggcttatctgcgatagcagggtgcttgagaggtacatcctggaagctaaagaagccgaaaacgtgaccatgggctgcgccgagggccctaggctcagtgaaaacattactgttcccgatacgaaagtcaatttctacgcctggaagcggatggaagtggaggaacaggccatagaggtgtggcaaggtctgtctctcctgagcgaggcaatccttcaagcccaggctctgctggccaattcaagccagccacccgagaccctccagctgcacattgacaaggctatcagcggtctgagatccctgacgtccctgttgcgagtcctgggcgctcagaaggagctgatgagtccacccgataccacacctccagcaccgctccgcacactcactgtggacaccttttgtaaactgttcagagtctacgccaactttctgcgaggcaagctgaagctctatacaggagaggtgtgtaggagaggagaccggtga

SEQ ID NO: 6 - DNA, 579 bp, GC-maximized sequence
atgggcgtgcccgagcggccgaccctgctcctgctgctcagcctgctgctcatccccctggggctgcccgtcctctgcgcccccccgcgcctgatctgcgactcccgggtgctggagcgctacatcctcgaggccaaggaggcggagaacgtgaccatgggctgcgccgaggggccccggctgagcgagaacatcacggtccccgacaccaaggtgaacttctacgcctggaagcgcatggaggtggaggagcaggccatcgaggtctggcagggcctgtccctcctgagcgaggccatcctgcaggcgcaggccctcctggccaactccagccagcccccggagacactgcagctccacatcgacaaggccatctccgggctgcggagcctgacctccctcctgcgcgtgctgggcgcgcagaaggagctcatgagcccgcccgacacgacccccccggccccgctgcggaccctgaccgtggacacgttctgcaagctcttccgcgtctacgccaacttcctgcggggcaagctgaagctctacaccggggaggtgtgccgccggggcgaccgctga

SEQ ID NO: 7 - RNA, 579 nt, Mus musculus
augggggugcccgaacgucccacccugcugcuuuuacucuccuugcuacugauuccucugggccucccaguccucugugcucccccacgccucaucugcgacagucgaguucuggagagguacaucuuagaggccaaggaggcagaaaaugucacgauggguugugcagaaggucccagacugagugaaaauauuacagucccagauaccaaagucaacuucuaugcuuggaaaagaauggagguggaagaacaggccauagaaguuuggcaaggccugucccugcucucagaagccauccugcaggcccaggcccugcuagccaauuccucccagccaccagagacccuucagcuucauauagacaaagccaucaguggucuacguagccucacuucacugcuucggguacugggagcucagaaggaauugaugucgccuccagauaccaccccaccugcuccacuccgaacacucacaguggauacuuucugcaagcucuuccgggucuacgccaacuuccuccgggggaaacugaagcuguacacgggagaggucugcaggagaggggacagguga

SEQ ID NO: 8 - RNA, 579 nt, Artificial Sequence
  GC-rich sequence
augggcguccccgaaaggccuacccugcugcugcuccugucucugcuccugaucccccugggacugcccgugcugugcgccccucccaggcugaucugcgacagcagggugcuggaaagauacauccuggaagccaaagaggccgagaacgucacaaugggcugcgccgagggccccagacugagcgagaacaucaccgugcccgacaccaaggucaacuucuacgccuggaagaggauggaaguggaggaacaggccaucgaggucuggcagggacugucucugcuguccgaggccauccugcaggcccaggcucugcuggccaauucuagccagccccccgagacacugcagcugcacaucgacaaggccaucagcggccugagaagccugaccagccugcugagggugcugggagcccagaaagagcugaugagccccccugacaccacccccccugccccccugaggacccugaccguggacaccuucugcaagcuguucaggguguacgccaacuuccugaggggcaagcugaagcuguacaccggcgaggucugcagacggggcgacagauga

SEQ ID NO: 9 - RNA, 579 nt, Artificial Sequence
  A-rich sequence
augggagugccagaaagaccaacccugcugcugcugcucagccugcuacugaucccacugggacucccaguccucugcgcaccaccaagacucaucugcgacagcagagugcuggaaagauacauccuagaagcaaaagaagcagaaaacgucacgaugggaugcgcagaaggaccaagacugagcgaaaacaucacagucccagacaccaaagucaacuucuacgcauggaaaagaauggaaguggaagaacaggcaauagaaguguggcaaggacugagccugcucagcgaagcaauccugcaggcacaggcacugcuagcaaacagcagccagccaccagaaacccugcagcugcacauagacaaagcaaucagcggacuaagaagccucaccagccugcugagaguacugggagcacagaaagaacugaugagcccaccagacaccaccccaccagcaccacucagaacacucacaguggacacuuucugcaaacucuucagagucuacgcaaacuuccucagaggaaaacugaaacuguacacgggagaagucugcagaagaggggacagauga

SEQ ID NO: 10 - RNA, 10 nt, Artificial Sequence
  Linker
gcauaugacu

SEQ ID NO: 11 - protein, 206 aa, Canis familiaris
MCEPAPPKPTQSAWHSFPECPALLLLLSLLLLPLGLPVLGAPPRLICDSRVLERYILEAREAENVTMGCAQGCSFSENITVPDTKVNFYTWKRMDVGQQALEVWQGLALLSEAILRGQALLANASQPSETPQLHVDKAVSSLRSLTSLLRALGAQKEAMSLPEEASPAPLRTFTVDTLCKLFRIYSNFLRGKLTLYTGEACRRGDR

SEQ ID NO: 12 - DNA, 621 bp, Canis familiaris
atgtgcgaacccgccccacctaagcccactcagtctgcttggcacagtttccccgaatgtccagctctcctgctgctgctctccctgctgctcctgcccctcgggctgcctgtgctgggcgctcctccaagactcatctgcgacagcagggtgctggagcggtacatcctggaggctagagaagccgagaatgtcaccatggggtgtgctcagggatgctccttcagcgagaacatcaccgtgcccgacactaaggtgaacttctatacatggaagcggatggatgtgggacagcaggccctcgaagtgtggcagggcctcgctctgctgtctgaagccatcctgaggggacaggccctcctggctaatgccagccagccttcagagaccccccagctgcacgtggacaaagccgtgtcaagcctgagatccctcacaagcctcctgagggctctgggcgctcagaaggaagccatgtctctgccagaggaagccagccctgccccactcaggaccttcactgtcgataccctgtgcaagctgttcaggatctattccaactttctgaggggcaaactgacactctatactggggaggcttgtaggcggggagaccgatga

SEQ ID NO: 13 - DNA, 621 bp, Artificial Sequence
  A-rich sequence
atgtgcgaaccagcaccacctaaaccaacacagagcgcatggcacagcttcccagaatgcccagcactgctgctgctgctcagcctgctactgctgccactgggactcccagtcctcggagcaccaccaagactcatctgcgacagcagagtgctggaaagatacatcctagaagcaagagaagcagaaaacgtcacgatgggatgcgcacaaggatgcagcttcagcgaaaacatcacagtcccagacaccaaagtcaacttctacacatggaaaagaatggacgtgggacagcaggcactggaagtgtggcaaggactggcactgctcagcgaagcaatcctgagaggacaggcactgctagcaaacgcaagccagccaagcgaaaccccacagctgcacgtagacaaagcagtgagcagcctaagaagcctcaccagcctgctgagagcactgggagcacagaaagaagccatgagcctgccagaagaagccagcccagcaccactcagaacattcacagtggacaccctgtgcaaactgttcagaatatacagcaacttcctcagaggaaaactgacactgtacacgggagaagcttgcagaggaggagacagatga

SEQ ID NO: 14 - RNA, 621 nt, Canis familiaris
augugcgaacccgccccaccuaagcccacucagucugcuuggcacaguuuccccgaauguccagcucuccugcugcugcucucccugcugcuccugccccucgggcugccugugcugggcgcuccuccaagacucaucugcgacagcagggugcuggagcgguacauccuggaggcuagagaagccgagaaugucaccauggggugugcucagggaugcuccuucagcgagaacaucaccgugcccgacacuaaggugaacuucuauacauggaagcggauggaugugggacagcaggcccucgaaguguggcagggccucgcucugcugucugaagccauccugaggggacaggcccuccuggcuaaugccagccagccuucagagaccccccagcugcacguggacaaagccgugucaagccugagaucccucacaagccuccugagggcucugggcgcucagaaggaagccaugucucugccagaggaagccagcccugccccacucaggaccuucacugucgauacccugugcaagcuguucaggaucuauuccaacuuucugaggggcaaacugacacucuauacuggggaggcuuguaggcggggagaccgauga

SEQ ID NO: 15 - RNA, 621 nt, Artificial Sequence
  A-rich sequence
augugcgaaccagcaccaccuaaaccaacacagagcgcauggcacagcuucccagaaugcccagcacugcugcugcugcucagccugcuacugcugccacugggacucccaguccucggagcaccaccaagacucaucugcgacagcagagugcuggaaagauacauccuagaagcaagagaagcagaaaacgucacgaugggaugcgcacaaggaugcagcuucagcgaaaacaucacagucccagacaccaaagucaacuucuacacauggaaaagaauggacgugggacagcaggcacuggaaguguggcaaggacuggcacugcucagcgaagcaauccugagaggacaggcacugcuagcaaacgcaagccagccaagcgaaaccccacagcugcacguagacaaagcagugagcagccuaagaagccucaccagccugcugagagcacugggagcacagaaagaagccaugagccugccagaagaagccagcccagcaccacucagaacauucacaguggacacccugugcaaacuguucagaauauacagcaacuuccucagaggaaaacugacacuguacacgggagaagcuugcagaggaggagacagauga